European Patent Application EP 4 574 211 A2, published June 25, 2025. Title: COMPOSITIONS OF GROWTH FACTOR FOR THE TREATMENT OF EYE DISEASE. Applicant: Claris Biotherapeutics, Inc. Application EP, filed May 13, 2022. The sequence listing filed with the application follows.

SEQUENCE LISTING (37 sequences)

SEQ ID NO: 1 - protein, 723 aa, Homo sapiens
MWVTKLLPALLLQHVLLHLLLLPIAIPYAEGQRKRRNTIHEFKKSAKTTLIKIDPALKIKTKKVNTADQCANRCTRNKGLPFTCKAFVFDKARKQCLWFPFNSMSSGVKKEFGHEFDLYENKDYIRNCIIGKGRSYKGTVSITKSGIKCQPWSSMIPHEHSYRGKDLQENYCRNPRGEEGGPWCFTSNPEVRYEVCDIPQCSEVECMTCNGESYRGLMDHTESGKICQRWDHQTPHRHKFLPERYPDKGFDDNYCRNPDGQPRPWCYTLDPHTRWEYCAIKTCADNTMNDTDVPLETTECIQGQGEGYRGTVNTIWNGIPCQRWDSQYPHEHDMTPENFKCKDLRENYCRNPDGSESPWCFTTDPNIRVGYCSQIPNCDMSHGQDCYRGNGKNYMGNLSQTRSGLTCSMWDKNMEDLHRHIFWEPDASKLNENYCRNPDDDAHGPWCYTGNPLIPWDYCPISRCEGDTTPTIVNLDHPVISCAKTKQLRVVNGIPTRTNIGWMVSLRYRNKHICGGSLIKESWVLTARQCFPSRDLKDYEAWLGIHDVHGRGDEKCKQVLNVSQLVYGPEGSDLVLMKLARPAVLDDFVSTIDLPNYGCTIPEKTSCSVYGWGYTGLINYDGLLRVAHLYIMGNEKCSQHHRGKVTLNESEICAGAEKIGSGPCEGDYGGPLVCEQHKMRMVLGVIVPGRGCAIPNRPGIFVRVAYYAKWIHKIILTYKVPQS

SEQ ID NO: 2 - protein, 728 aa, Homo sapiens
MWVTKLLPALLLQHVLLHLLLLPIAIPYAEGQRKRRNTIHEFKKSAKTTLIKIDPALKIKTKKVNTADQCANRCTRNKGLPFTCKAFVFDKARKQCLWFPFNSMSSGVKKEFGHEFDLYENKDYIRNCIIGKGRSYKGTVSITKSGIKCQPWSSMIPHEHSFLPSSYRGKDLQENYCRNPRGEEGGPWCFTSNPEVRYEVCDIPQCSEVECMTCNGESYRGLMDHTESGKICQRWDHQTPHRHKFLPERYPDKGFDDNYCRNPDGQPRPWCYTLDPHTRWEYCAIKTCADNTMNDTDVPLETTECIQGQGEGYRGTVNTIWNGIPCQRWDSQYPHEHDMTPENFKCKDLRENYCRNPDGSESPWCFTTDPNIRVGYCSQIPNCDMSHGQDCYRGNGKNYMGNLSQTRSGLTCSMWDKNMEDLHRHIFWEPDASKLNENYCRNPDDDAHGPWCYTGNPLIPWDYCPISRCEGDTTPTIVNLDHPVISCAKTKQLRVVNGIPTRTNIGWMVSLRYRNKHICGGSLIKESWVLTARQCFPSRDLKDYEAWLGIHDVHGRGDEKCKQVLNVSQLVYGPEGSDLVLMKLARPAVLDDFVSTIDLPNYGCTIPEKTSCSVYGWGYTGLINYDGLLRVAHLYIMGNEKCSQHHRGKVTLNESEICAGAEKIGSGPCEGDYGGPLVCEQHKMRMVLGVIVPGRGCAIPNRPGIFVRVAYYAKWIHKIILTYKVPQS

SEQ ID NO: 3 - protein, 290 aa, Homo sapiens
MWVTKLLPALLLQHVLLHLLLLPIAIPYAEGQRKRRNTIHEFKKSAKTTLIKIDPALKIKTKKVNTADQCANRCTRNKGLPFTCKAFVFDKARKQCLWFPFNSMSSGVKKEFGHEFDLYENKDYIRNCIIGKGRSYKGTVSITKSGIKCQPWSSMIPHEHSFLPSSYRGKDLQENYCRNPRGEEGGPWCFTSNPEVRYEVCDIPQCSEVECMTCNGESYRGLMDHTESGKICQRWDHQTPHRHKFLPERYPDKGFDDNYCRNPDGQPRPWCYTLDPHTRWEYCAIKTCET

SEQ ID NO: 4 - protein, 296 aa, Homo sapiens
MWVTKLLPALLLQHVLLHLLLLPIAIPYAEGQRKRRNTIHEFKKSAKTTLIKIDPALKIKTKKVNTADQCANRCTRNKGLPFTCKAFVFDKARKQCLWFPFNSMSSGVKKEFGHEFDLYENKDYIRNCIIGKGRSYKGTVSITKSGIKCQPWSSMIPHEHSFLPSSYRGKDLQENYCRNPRGEEGGPWCFTSNPEVRYEVCDIPQCSEVECMTCNGESYRGLMDHTESGKICQRWDHQTPHRHKFLPERYPDKGFDDNYCRNPDGQPRPWCYTLDPHTRWEYCAIKNMRDITWALN

SEQ ID NO: 5 - protein, 285 aa, Homo sapiens
MWVTKLLPALLLQHVLLHLLLLPIAIPYAEGQRKRRNTIHEFKKSAKTTLIKIDPALKIKTKKVNTADQCANRCTRNKGLPFTCKAFVFDKARKQCLWFPFNSMSSGVKKEFGHEFDLYENKDYIRNCIIGKGRSYKGTVSITKSGIKCQPWSSMIPHEHSYRGKDLQENYCRNPRGEEGGPWCFTSNPEVRYEVCDIPQCSEVECMTCNGESYRGLMDHTESGKICQRWDHQTPHRHKFLPERYPDKGFDDNYCRNPDGQPRPWCYTLDPHTRWEYCAIKTCET

SEQ ID NO: 6 - protein, 210 aa, Homo sapiens
MWVTKLLPALLLQHVLLHLLLLPIAIPYAEGQRKRRNTIHEFKKSAKTTLIKIDPALKIKTKKVNTADQCANRCTRNKGLPFTCKAFVFDKARKQCLWFPFNSMSSGVKKEFGHEFDLYENKDYIRNCIIGKGRSYKGTVSITKSGIKCQPWSSMIPHEHSFLPSSYRGKDLQENYCRNPRGEEGGPWCFTSNPEVRYEVCDIPQCSEGK

SEQ ID NO: 7 - protein, 728 aa, synthetic construct
  REGION 1..728: note = HGF Variant
MWVTKLLPALLLQHVLLHLLLLPIAIPYAEGQRKRRNTIHEFKKSAKTTLIKIDPALEIKTKKANTADQCANRCTRSKGLPFTCKAFVFDKARKRCLWFPFNSMSSGVKKEFGHEFDLYENKDYIRDCIIGKGRSYRGTVSITKSGIKCQPWSAMIPHEHSFLPSSYRGEDLRENYCRNPRGEEGGPWCYTSDPEVRYEVCDIPQCSEVECMTCNGESYRGLMDHTESGKICQRWDHQTPHRHKFLPERYPDKGFDDNYCRNPDGQPRPWCYTLDPHTRWEYCAIKTCADNTMNDTDVPLETTECIQGQGEGYRGTVNTIWNGIPCQRWDSQYPHEHDMTPENFKCKDLRENYCRNPDGSESPWCFTTDPNIRVGYCSQIPNCDMSHGQDCYRGNGKNYMGNLSQTRSGLTCSMWDKNMEDLHRHIFWEPDASKLNENYCRNPDDDAHGPWCYTGNPLIPWDYCPISRCEGDTTPTIVNLDHPVISCAKTKQLRVVNGIPTRTNIGWMVSLRYRNKHICGGSLIKESWVLTARQCFPSRDLKDYEAWLGIHDVHGRGDEKCKQVLNVSQLVYGPEGSDLVLMKLARPAVLDDFVSTIDLPNYGCTIPEKTSCSVYGWGYTGLINYDGLLRVAHLYIMGNEKCSQHHRGKVTLNESEICAGAEKIGSGPCEGDYGGPLVCEQHKMRMVLGVIVPGRGCAIPNRPGIFVRVAYYAKWIHKIILTYKVPQS

SEQ ID NO: 8 - protein, 728 aa, synthetic construct
  REGION 1..728: note = HGF Variant
MWVTKLLPALLLQHVLLHLLLLPIAIPYAEGQRKRRNTIHEFKKSAKTTLIKIDPALKIKTEKANTADQCANRCIRNKGLPFTCKAFVFDKARKRCLWFPVNSMSSGVKKEFGHEFDLYENKDYTRNCIVGNGRSYRGTVSTTKSGIKCQPWSAMIPHEHSFLPSSYRGEDLRENYCRNPRGEEGGPWCYTSDPEVRYEVCDIPQCSEVECMTCNGESYRGLMDHTESGKICQRWDHQTPHRHKFLPERYPDKGFDDNYCRNPDGQPRPWCYTLDPHTRWEYCAIKTCADNTMNDTDVPLETTECIQGQGEGYRGTVNTIWNGIPCQRWDSQYPHEHDMTPENFKCKDLRENYCRNPDGSESPWCFTTDPNIRVGYCSQIPNCDMSHGQDCYRGNGKNYMGNLSQTRSGLTCSMWDKNMEDLHRHIFWEPDASKLNENYCRNPDDDAHGPWCYTGNPLIPWDYCPISRCEGDTTPTIVNLDHPVISCAKTKQLRVVNGIPTRTNIGWMVSLRYRNKHICGGSLIKESWVLTARQCFPSRDLKDYEAWLGIHDVHGRGDEKCKQVLNVSQLVYGPEGSDLVLMKLARPAVLDDFVSTIDLPNYGCTIPEKTSCSVYGWGYTGLINYDGLLRVAHLYIMGNEKCSQHHRGKVTLNESEICAGAEKIGSGPCEGDYGGPLVCEQHKMRMVLGVIVPGRGCAIPNRPGIFVRVAYYAKWIHKIILTYKVPQS

SEQ ID NO: 9 - protein, 728 aa, synthetic construct
  REGION 1..728: note = HGF Variant
MWVTKLLPALLLQHVLLHLLLLPIAIPYAEGQRKRRNTIHEFKKSAKTTLIKIDPALKIKTEKANTADQCANRCTRSKGLPFTCKAFVFDKARKRCLWFPFNSMSSGVKKEFGHEFDLYENKDYIRDCIVGNGRSYRGTVSITKSGIECQPWSAMIPHEHSFLPSSYRGEDLRENYCRNPRGEEGGPWCYTSDPEVRYEVCDIPQCSEVECMTCNGESYRGLMDHTESGKICQRWDHQTPHRHKFLPERYPDKGFDDNYCRNPDGQPRPWCYTLDPHTRWEYCAIKTCADNTMNDTDVPLETTECIQGQGEGYRGTVNTIWNGIPCQRWDSQYPHEHDMTPENFKCKDLRENYCRNPDGSESPWCFTTDPNIRVGYCSQIPNCDMSHGQDCYRGNGKNYMGNLSQTRSGLTCSMWDKNMEDLHRHIFWEPDASKLNENYCRNPDDDAHGPWCYTGNPLIPWDYCPISRCEGDTTPTIVNLDHPVISCAKTKQLRVVNGIPTRTNIGWMVSLRYRNKHICGGSLIKESWVLTARQCFPSRDLKDYEAWLGIHDVHGRGDEKCKQVLNVSQLVYGPEGSDLVLMKLARPAVLDDFVSTIDLPNYGCTIPEKTSCSVYGWGYTGLINYDGLLRVAHLYIMGNEKCSQHHRGKVTLNESEICAGAEKIGSGPCEGDYGGPLVCEQHKMRMVLGVIVPGRGCAIPNRPGIFVRVAYYAKWIHKIILTYKVPQS

SEQ ID NO: 10 - protein, 728 aa, synthetic construct
  REGION 1..728: note = HGF Variant
MWVTKLLPALLLQHVLLHLLLLPIAIPYAKGQGKRRNTIHEFKKSAKTTLIKIDPALKIKTEKADTADQCANRCTRSKGLPFTCKAFVFDKARKQCLWFPFNSMSSGVKKEFGHEFDLYENKDYIRDCIVGNGRSYRGTVSVTKSGIKCQPWSSMIPHEHSFLPSSYRGEDLRENYCRNPRGEEGGPWCYTSDPEVRYEVCDIPQCSEVECMTCNGESYRGLMDHTESGKICQRWDHQTPHRHKFLPERYPDKGFDDNYCRNPDGQPRPWCYTLDPHTRWEYCAIKTCADNTMNDTDVPLETTECIQGQGEGYRGTVNTIWNGIPCQRWDSQYPHEHDMTPENFKCKDLRENYCRNPDGSESPWCFTTDPNIRVGYCSQIPNCDMSHGQDCYRGNGKNYMGNLSQTRSGLTCSMWDKNMEDLHRHIFWEPDASKLNENYCRNPDDDAHGPWCYTGNPLIPWDYCPISRCEGDTTPTIVNLDHPVISCAKTKQLRVVNGIPTRTNIGWMVSLRYRNKHICGGSLIKESWVLTARQCFPSRDLKDYEAWLGIHDVHGRGDEKCKQVLNVSQLVYGPEGSDLVLMKLARPAVLDDFVSTIDLPNYGCTIPEKTSCSVYGWGYTGLINYDGLLRVAHLYIMGNEKCSQHHRGKVTLNESEICAGAEKIGSGPCEGDYGGPLVCEQHKMRMVLGVIVPGRGCAIPNRPGIFVRVAYYAKWIHKIILTYKVPQS

SEQ ID NO: 11 - protein, 728 aa, synthetic construct
  REGION 1..728: note = HGF Variant
MWVTKLLPALLLQHVLLHLLLLPIAIPYAEGQRKRRNAIHEFKKSAKATLIKIDPALKIKTEKANTADQCANRCTRSKGLPFTCKAFVFDKARKRCLWFPFNSMSSGVKKEFGHEFDLYENKDYIRDCIVGNGRSYRGTVSITKSGIECQPWSSMIPHEHSFLPSSYRGEDLQENYCRNPWGEEGGPWCYTSDPEVRYEVCDIPQCSEVECMTCNGESYRGLMDHTESGKICQRWDHQTPHRHKFLPERYPDKGFDDNYCRNPDGQPRPWCYTLDPHTRWEYCAIKTCADNTMNDTDVPLETTECIQGQGEGYRGTVNTIWNGIPCQRWDSQYPHEHDMTPENFKCKDLRENYCRNPDGSESPWCFTTDPNIRVGYCSQIPNCDMSHGQDCYRGNGKNYMGNLSQTRSGLTCSMWDKNMEDLHRHIFWEPDASKLNENYCRNPDDDAHGPWCYTGNPLIPWDYCPISRCEGDTTPTIVNLDHPVISCAKTKQLRVVNGIPTRTNIGWMVSLRYRNKHICGGSLIKESWVLTARQCFPSRDLKDYEAWLGIHDVHGRGDEKCKQVLNVSQLVYGPEGSDLVLMKLARPAVLDDFVSTIDLPNYGCTIPEKTSCSVYGWGYTGLINYDGLLRVAHLYIMGNEKCSQHHRGKVTLNESEICAGAEKIGSGPCEGDYGGPLVCEQHKMRMVLGVIVPGRGCAIPNRPGIFVRVAYYAKWIHKIILTYKVPQS

SEQ ID NO: 12 - protein, 728 aa, synthetic construct
  REGION 1..728: note = HGF Variant
MWVTKLLPALLLQHVLLHLLLLPIAIPYAEGQRKRRNTIHEFKKSAKTTLIKIDPALKIKTEKANTADQCANRCTRSKGLPFTCKAFVFDKARKRCLWFPFNSMSSGVKKEFGHEFDLYENKDYTRNCIVGNGRSYRGTVSITKSGIECQPWSAMIPHEHSFLPSSYQGEDLRENYCRNPRGEEGGPWCYTSDPEVRYEVCDIPQCSEVECMTCNGESYRGLMDHTESGKICQRWDHQTPHRHKFLPERYPDKGFDDNYCRNPDGQPRPWCYTLDPHTRWEYCAIKTCADNTMNDTDVPLETTECIQGQGEGYRGTVNTIWNGIPCQRWDSQYPHEHDMTPENFKCKDLRENYCRNPDGSESPWCFTTDPNIRVGYCSQIPNCDMSHGQDCYRGNGKNYMGNLSQTRSGLTCSMWDKNMEDLHRHIFWEPDASKLNENYCRNPDDDAHGPWCYTGNPLIPWDYCPISRCEGDTTPTIVNLDHPVISCAKTKQLRVVNGIPTRTNIGWMVSLRYRNKHICGGSLIKESWVLTARQCFPSRDLKDYEAWLGIHDVHGRGDEKCKQVLNVSQLVYGPEGSDLVLMKLARPAVLDDFVSTIDLPNYGCTIPEKTSCSVYGWGYTGLINYDGLLRVAHLYIMGNEKCSQHHRGKVTLNESEICAGAEKIGSGPCEGDYGGPLVCEQHKMRMVLGVIVPGRGCAIPNRPGIFVRVAYYAKWIHKIILTYKVPQS

SEQ ID NO: 13 - protein, 728 aa, synthetic construct; identical to SEQ ID NO: 2
  REGION 1..728: note = HGF Variant

SEQ ID NO: 14 - protein, 728 aa, synthetic construct
  REGION 1..728: note = HGF Variant
MWVTKLLPALLLQHVLLHLLLLPIAIPYAEGQRKRRDAIHECKRSAKTTLIKIDPALKIKTEKANTADQCANRCTRNKGLPSTCKAFVFDKARKRRLRFPFNSMSSGVKKEFGHEFDLYENKDYTRNCIVGKGRSYRGTVSTTKSGIKCQPWSAMIPHEHSFLPSSYRGEDLRENYCRNPRGEEGGPWCYTSDPEVRYEVCDIPQCSEVECMTCNGESYRGLMDHTESGKICQRWDHQTPHRHKFLPERYPDKGFDDNYCRNPDGQPRPWCYTLDPHTRWEYCAIKTCADNTMNDTDVPLETTECIQGQGEGYRGTVNTIWNGIPCQRWDSQYPHEHDMTPENFKCKDLRENYCRNPDGSESPWCFTTDPNIRVGYCSQIPNCDMSHGQDCYRGNGKNYMGNLSQTRSGLTCSMWDKNMEDLHRHIFWEPDASKLNENYCRNPDDDAHGPWCYTGNPLIPWDYCPISRCEGDTTPTIVNLDHPVISCAKTKQLRVVNGIPTRTNIGWMVSLRYRNKHICGGSLIKESWVLTARQCFPSRDLKDYEAWLGIHDVHGRGDEKCKQVLNVSQLVYGPEGSDLVLMKLARPAVLDDFVSTIDLPNYGCTIPEKTSCSVYGWGYTGLINYDGLLRVAHLYIMGNEKCSQHHRGKVTLNESEICAGAEKIGSGPCEGDYGGPLVCEQHKMRMVLGVIVPGRGCAIPNRPGIFVRVAYYAKWIHKIILTYKVPQS

SEQ ID NO: 15 - protein, 728 aa, synthetic construct
  REGION 1..728: note = HGF Variant
MWVTKLLPALLLQHVLLHLLLLPIAIPYAEGQGKRRNTIHEFKKSAKTTLIKIDPALKIKTEKVNTADQCANRCTRSKGLPFTCKAFVFDKARKRCLWFPFNSMSSGVKKEFGHEFDLYENKDYIRDCIIGRGRSYRGTVSITKSGIKCQPWSAMIPHEHSFLPSSYRGEDLRENYCRNPRGEEGGPWCYTSDPEVRYEVCDIPQCSEVECMTCNGESYRGLMDHTESGKICQRWDHQTPHRHKFLPERYPDKGFDDNYCRNPDGQPRPWCYTLDPHTRWEYCAIKTCADNTMNDTDVPLETTECIQGQGEGYRGTVNTIWNGIPCQRWDSQYPHEHDMTPENFKCKDLRENYCRNPDGSESPWCFTTDPNIRVGYCSQIPNCDMSHGQDCYRGNGKNYMGNLSQTRSGLTCSMWDKNMEDLHRHIFWEPDASKLNENYCRNPDDDAHGPWCYTGNPLIPWDYCPISRCEGDTTPTIVNLDHPVISCAKTKQLRVVNGIPTRTNIGWMVSLRYRNKHICGGSLIKESWVLTARQCFPSRDLKDYEAWLGIHDVHGRGDEKCKQVLNVSQLVYGPEGSDLVLMKLARPAVLDDFVSTIDLPNYGCTIPEKTSCSVYGWGYTGLINYDGLLRVAHLYIMGNEKCSQHHRGKVTLNESEICAGAEKIGSGPCEGDYGGPLVCEQHKMRMVLGVIVPGRGCAIPNRPGIFVRVAYYAKWIHKIILTYKVPQS

SEQ ID NO: 16 - protein, 728 aa, synthetic construct
  REGION 1..728: note = HGF Variant
MWVTKLLPALLLQHVLLHLLLLPIAIPHAEGQRKRRNTIHEFKKSAKTTLIKIDPALKIKTEKANTADQCANRCTRSKGLPFTCKAFVFDKARKRCLWFPFNSMSSGVKKEFGHEFDLYENKDYTRNCIVGNGRSYRGTVSTTKSGIKCQPWSAMIPHEHSFLPSSYRGEDLRENYCRNPRGEEGGPWCYTSDPEVRYEVCDIPQCSEVECMTCNGESYRGLMDHTESGKICQRWDHQTPHRHKFLPERYPDKGFDDNYCRNPDGQPRPWCYTLDPHTRWEYCAIKTCADNTMNDTDVPLETTECIQGQGEGYRGTVNTIWNGIPCQRWDSQYPHEHDMTPENFKCKDLRENYCRNPDGSESPWCFTTDPNIRVGYCSQIPNCDMSHGQDCYRGNGKNYMGNLSQTRSGLTCSMWDKNMEDLHRHIFWEPDASKLNENYCRNPDDDAHGPWCYTGNPLIPWDYCPISRCEGDTTPTIVNLDHPVISCAKTKQLRVVNGIPTRTNIGWMVSLRYRNKHICGGSLIKESWVLTARQCFPSRDLKDYEAWLGIHDVHGRGDEKCKQVLNVSQLVYGPEGSDLVLMKLARPAVLDDFVSTIDLPNYGCTIPEKTSCSVYGWGYTGLINYDGLLRVAHLYIMGNEKCSQHHRGKVTLNESEICAGAEKIGSGPCEGDYGGPLVCEQHKMRMVLGVIVPGRGCAIPNRPGIFVRVAYYAKWIHKIILTYKVPQS

SEQ ID NO: 17 - protein, 728 aa, synthetic construct
  REGION 1..728: note = HGF Variant
MWVTKLLPALLLQHVLLHLLLLPIAIPYAEGQRKRRNTIHEFKKSAKTTLIKIDPALKIKTEKANTADQCANRCTRSRGLPFTCKAFVFDKARKQCLWFPFNSMSSGVKKEFGHEFDLYENKDYIRDCIIGNGRSYRGTVSVTKSGIKCQPWSAMIPHEHSFLPSSYRGEDLRENYCRNPRGEEGGPWCYTSDPEVRYEVCDIPQCSEVECMTCNGESYRGLMDHTESGKICQRWDHQTPHRHKFLPERYPDKGFDDNYCRNPDGQPRPWCYTLDPHTRWEYCAIKTCADNTMNDTDVPLETTECIQGQGEGYRGTVNTIWNGIPCQRWDSQYPHEHDMTPENFKCKDLRENYCRNPDGSESPWCFTTDPNIRVGYCSQIPNCDMSHGQDCYRGNGKNYMGNLSQTRSGLTCSMWDKNMEDLHRHIFWEPDASKLNENYCRNPDDDAHGPWCYTGNPLIPWDYCPISRCEGDTTPTIVNLDHPVISCAKTKQLRVVNGIPTRTNIGWMVSLRYRNKHICGGSLIKESWVLTARQCFPSRDLKDYEAWLGIHDVHGRGDEKCKQVLNVSQLVYGPEGSDLVLMKLARPAVLDDFVSTIDLPNYGCTIPEKTSCSVYGWGYTGLINYDGLLRVAHLYIMGNEKCSQHHRGKVTLNESEICAGAEKIGSGPCEGDYGGPLVCEQHKMRMVLGVIVPGRGCAIPNRPGIFVRVAYYAKWIHKIILTYKVPQS

SEQ ID NO: 18 - protein, 728 aa, synthetic construct
  REGION 1..728: note = HGF Variant
MWVTKLLPALLLQHVLLHLLLLPIAIPYAEGQRKRRNTIHEFKKSAKTTLIKIDPALKIKTEKANTADQCANRCTRNKGLPFTCKAFVFDKARKRCLWFPFNSMSSGVKKEFGHEFDLYENKDYIRDCIVGNGRSYRGTVSITKSGIKCQPWSSMIPHEHSFLPSSYRGEDLRENYCRNPRGEEGGPWCYTSDPEVRYEVCDIPQCSEVECMTCNGESYRGLMDHTESGKICQRWDHQTPHRHKFLPERYPDKGFDDNYCRNPDGQPRPWCYTLDPHTRWEYCAIKTCADNTMNDTDVPLETTECIQGQGEGYRGTVNTIWNGIPCQRWDSQYPHEHDMTPENFKCKDLRENYCRNPDGSESPWCFTTDPNIRVGYCSQIPNCDMSHGQDCYRGNGKNYMGNLSQTRSGLTCSMWDKNMEDLHRHIFWEPDASKLNENYCRNPDDDAHGPWCYTGNPLIPWDYCPISRCEGDTTPTIVNLDHPVISCAKTKQLRVVNGIPTRTNIGWMVSLRYRNKHICGGSLIKESWVLTARQCFPSRDLKDYEAWLGIHDVHGRGDEKCKQVLNVSQLVYGPEGSDLVLMKLARPAVLDDFVSTIDLPNYGCTIPEKTSCSVYGWGYTGLINYDGLLRVAHLYIMGNEKCSQHHRGKVTLNESEICAGAEKIGSGPCEGDYGGPLVCEQHKMRMVLGVIVPGRGCAIPNRPGIFVRVAYYAKWIHKIILTYKVPQS

SEQ ID NO: 19 - protein, 728 aa, synthetic construct
  REGION 1..728: note = HGF Variant
MWVTKLLPALLLQHVLLHLLLLPIAIPYAEGQRKRRNTIHEFKKSVKTTLIKIDPALKIKTEKANTADQCANRCTRSKGLPFTCKAFVFDKARKRCLWFPVNSMSSGVKKESGHEFDLYENKDYIRDCIVGNGRSYRGTVSTTKSGIKCQPWSAMIPHEHSFLPSSYRGEDLRENYCRNPRGEEGGPWCYTSDPEVRYEVCDIPQCSEVECMTCNGESYRGLMDHTESGKICQRWDHQTPHRHKFLPERYPDKGFDDNYCRNPDGQPRPWCYTLDPHTRWEYCAIKTCADNTMNDTDVPLETTECIQGQGEGYRGTVNTIWNGIPCQRWDSQYPHEHDMTPENFKCKDLRENYCRNPDGSESPWCFTTDPNIRVGYCSQIPNCDMSHGQDCYRGNGKNYMGNLSQTRSGLTCSMWDKNMEDLHRHIFWEPDASKLNENYCRNPDDDAHGPWCYTGNPLIPWDYCPISRCEGDTTPTIVNLDHPVISCAKTKQLRVVNGIPTRTNIGWMVSLRYRNKHICGGSLIKESWVLTARQCFPSRDLKDYEAWLGIHDVHGRGDEKCKQVLNVSQLVYGPEGSDLVLMKLARPAVLDDFVSTIDLPNYGCTIPEKTSCSVYGWGYTGLINYDGLLRVAHLYIMGNEKCSQHHRGKVTLNESEICAGAEKIGSGPCEGDYGGPLVCEQHKMRMVLGVIVPGRGCAIPNRPGIFVRVAYYAKWIHKIILTYKVPQS

SEQ ID NO: 20 - protein, 728 aa, synthetic construct
  REGION 1..728: note = HGF Variant
MWVTKLLPALLLQHVLLHLLLLPIAIPYAEGQRKRRNTIHEFKKSAKTTLIKIDPALKIKTEKANTADQCANRCTRSKGLPFTCKAFVFDKARKRCLWFPFNSMSSGVKKEFGHEFDLYENKDYIRDCIVGNGRSYRGTVSITKSGIKCQPWSSMIPHEHSFLPSSYRGEDLRENYCRNPWGEEGGPWCYTSDPEVRYEVCDIPQCSEVECMTCNGESYRGLMDHTESGKICQRWDHQTPHRHKFLPERYPDKGFDDNYCRNPDGQPRPWCYTLDPHTRWEYCAIKTCADNTMNDTDVPLETTECIQGQGEGYRGTVNTIWNGIPCQRWDSQYPHEHDMTPENFKCKDLRENYCRNPDGSESPWCFTTDPNIRVGYCSQIPNCDMSHGQDCYRGNGKNYMGNLSQTRSGLTCSMWDKNMEDLHRHIFWEPDASKLNENYCRNPDDDAHGPWCYTGNPLIPWDYCPISRCEGDTTPTIVNLDHPVISCAKTKQLRVVNGIPTRTNIGWMVSLRYRNKHICGGSLIKESWVLTARQCFPSRDLKDYEAWLGIHDVHGRGDEKCKQVLNVSQLVYGPEGSDLVLMKLARPAVLDDFVSTIDLPNYGCTIPEKTSCSVYGWGYTGLINYDGLLRVAHLYIMGNEKCSQHHRGKVTLNESEICAGAEKIGSGPCEGDYGGPLVCEQHKMRMVLGVIVPGRGCAIPNRPGIFVRVAYYAKWIHKIILTYKVPQS

SEQ ID NO: 21 - protein, 728 aa, synthetic construct
  REGION 1..728: note = HGF Variant
MWVTKLLPALLLQHVLLHLLLLPIAIPYAEGQRKRRNTIHEFKKSAKTTLIKIDPALRIKTEKANTADQCANRCTRSRGLPFTCKAFVFDKARKRCLWFPFNSMSSGVKKEFGHEFDLYENKDYIRDCIIGNGRSYRGTVSITKSGIKCQPWSSMIPHEHSFLPSSYRGEDLRENYCRNPRGEEGGPWCYTSDPEVRYEVCDIPQCSEVECMTCNGESYRGLMDHTESGKICQRWDHQTPHRHKFLPERYPDKGFDDNYCRNPDGQPRPWCYTLDPHTRWEYCAIKTCADNTMNDTDVPLETTECIQGQGEGYRGTVNTIWNGIPCQRWDSQYPHEHDMTPENFKCKDLRENYCRNPDGSESPWCFTTDPNIRVGYCSQIPNCDMSHGQDCYRGNGKNYMGNLSQTRSGLTCSMWDKNMEDLHRHIFWEPDASKLNENYCRNPDDDAHGPWCYTGNPLIPWDYCPISRCEGDTTPTIVNLDHPVISCAKTKQLRVVNGIPTRTNIGWMVSLRYRNKHICGGSLIKESWVLTARQCFPSRDLKDYEAWLGIHDVHGRGDEKCKQVLNVSQLVYGPEGSDLVLMKLARPAVLDDFVSTIDLPNYGCTIPEKTSCSVYGWGYTGLINYDGLLRVAHLYIMGNEKCSQHHRGKVTLNESEICAGAEKIGSGPCEGDYGGPLVCEQHKMRMVLGVIVPGRGCAIPNRPGIFVRVAYYAKWIHKIILTYKVPQS

SEQ ID NO: 22 - protein, 728 aa, synthetic construct
  REGION 1..728: note = HGF Variant
MWVTKLLPALLLQHVLLHLLLLPIAIPYAEGQRKRRNTIHEFKKSAKTTLIKIDPALKIKTEKANTADQCANRCTRSRRLPFTCKAFVFDKARKRCLWFPFNSMSSGVKKEFGHEFDLYENKDYIRDCIIGKGRSYRGTVSVTKSGIECQPWSAMIPHEHSFLPSNYRGEDLRENYCRNPRGEEGGPWCYTSDPEVRYEVCDIPQCSEVECMTCNGESYRGLMDHTESGKICQRWDHQTPHRHKFLPERYPDKGFDDNYCRNPDGQPRPWCYTLDPHTRWEYCAIKTCADNTMNDTDVPLETTECIQGQGEGYRGTVNTIWNGIPCQRWDSQYPHEHDMTPENFKCKDLRENYCRNPDGSESPWCFTTDPNIRVGYCSQIPNCDMSHGQDCYRGNGKNYMGNLSQTRSGLTCSMWDKNMEDLHRHIFWEPDASKLNENYCRNPDDDAHGPWCYTGNPLIPWDYCPISRCEGDTTPTIVNLDHPVISCAKTKQLRVVNGIPTRTNIGWMVSLRYRNKHICGGSLIKESWVLTARQCFPSRDLKDYEAWLGIHDVHGRGDEKCKQVLNVSQLVYGPEGSDLVLMKLARPAVLDDFVSTIDLPNYGCTIPEKTSCSVYGWGYTGLINYDGLLRVAHLYIMGNEKCSQHHRGKVTLNESEICAGAEKIGSGPCEGDYGGPLVCEQHKMRMVLGVIVPGRGCAIPNRPGIFVRVAYYAKWIHKIILTYKVPQS

SEQ ID NO: 23 - protein, 728 aa, synthetic construct; identical to SEQ ID NO: 9
  REGION 1..728: note = HGF Variant

SEQ ID NO: 24 - protein, 728 aa, synthetic construct
  REGION 1..728: note = HGF Variant
MWVTKLLPALLLQHVLLHLLLLPIAIPYAEGQRKRRNTIHEFKKSAKTTLIKIDPALKIKTKKVDTADQCANRCTRNKGLPFTCKAFVFDKARKRCLWFPFNSMSSGVKKEFGHEFDLYENKDYIRDCIIGNGRSYRGTVSITKSGIKCQPWSSMIPHEHSFLPSSYRGEDLRENYCRNPRGEEGGPWCYTSDPEVRYEVCDIPQCSEVECMTCNGESYRGLMDHTESGKICQRWDHQTPHRHKFLPERYPDKGFDDNYCRNPDGQPRPWCYTLDPHTRWEYCAIKTCADNTMNDTDVPLETTECIQGQGEGYRGTVNTIWNGIPCQRWDSQYPHEHDMTPENFKCKDLRENYCRNPDGSESPWCFTTDPNIRVGYCSQIPNCDMSHGQDCYRGNGKNYMGNLSQTRSGLTCSMWDKNMEDLHRHIFWEPDASKLNENYCRNPDDDAHGPWCYTGNPLIPWDYCPISRCEGDTTPTIVNLDHPVISCAKTKQLRVVNGIPTRTNIGWMVSLRYRNKHICGGSLIKESWVLTARQCFPSRDLKDYEAWLGIHDVHGRGDEKCKQVLNVSQLVYGPEGSDLVLMKLARPAVLDDFVSTIDLPNYGCTIPEKTSCSVYGWGYTGLINYDGLLRVAHLYIMGNEKCSQHHRGKVTLNESEICAGAEKIGSGPCEGDYGGPLVCEQHKMRMVLGVIVPGRGCAIPNRPGIFVRVAYYAKWIHKIILTYKVPQS

SEQ ID NO: 25 - protein, 728 aa, synthetic construct
  REGION 1..728: note = HGF Variant
MWVTKLLPALLLQHVLLHLLLLPIAIPYAEGQGKRRNTIHEFKKSAKTTLIKIDPALRIKTEKANTADQCANRCTRSKGLPFTCKAFVFDKARKRCLWFPFNSMSSGVKKEFGHEFDLYENKAYIRDCIIGRGRNYRGTVSITKSGIKCQPWSAMIPHEHSFLPSSYRGEDLRENYCRNPRGEEGGPWCYTSDPEVRYEVCDIPQCSEVECMTCNGESYRGLMDHTESGKICQRWDHQTPHRHKFLPERYPDKGFDDNYCRNPDGQPRPWCYTLDPHTRWEYCAIKTCADNTMNDTDVPLETTECIQGQGEGYRGTVNTIWNGIPCQRWDSQYPHEHDMTPENFKCKDLRENYCRNPDGSESPWCFTTDPNIRVGYCSQIPNCDMSHGQDCYRGNGKNYMGNLSQTRSGLTCSMWDKNMEDLHRHIFWEPDASKLNENYCRNPDDDAHGPWCYTGNPLIPWDYCPISRCEGDTTPTIVNLDHPVISCAKTKQLRVVNGIPTRTNIGWMVSLRYRNKHICGGSLIKESWVLTARQCFPSRDLKDYEAWLGIHDVHGRGDEKCKQVLNVSQLVYGPEGSDLVLMKLARPAVLDDFVSTIDLPNYGCTIPEKTSCSVYGWGYTGLINYDGLLRVAHLYIMGNEKCSQHHRGKVTLNESEICAGAEKIGSGPCEGDYGGPLVCEQHKMRMVLGVIVPGRGCAIPNRPGIFVRVAYYAKWIHKIILTYKVPQS

SEQ ID NO: 26 - protein, 728 aa, synthetic construct
  REGION 1..728: note = HGF Variant
MWVTKLLPALLLQHVLLHLLLLPIAIPYAKGQRKRRNTIHEFKKSAKTTLIKIDPALEIKTEKVNTADQCANRCIRNKGLPFTCKAFVFDKARKRCLWFPFNSMSSGVKKEFGHEFDLYENKAYIRDCIIGRGRNYRGTVSITKSGIKCQPWSAMIPHEHSFLPSSYRGEDLRENYCRNPRGEEGGPWCYTSDPEVRYEVCDIPQCSEVECMTCNGESYRGLMDHTESGKICQRWDHQTPHRHKFLPERYPDKGFDDNYCRNPDGQPRPWCYTLDPHTRWEYCAIKTCADNTMNDTDVPLETTECIQGQGEGYRGTVNTIWNGIPCQRWDSQYPHEHDMTPENFKCKDLRENYCRNPDGSESPWCFTTDPNIRVGYCSQIPNCDMSHGQDCYRGNGKNYMGNLSQTRSGLTCSMWDKNMEDLHRHIFWEPDASKLNENYCRNPDDDAHGPWCYTGNPLIPWDYCPISRCEGDTTPTIVNLDHPVISCAKTKQLRVVNGIPTRTNIGWMVSLRYRNKHICGGSLIKESWVLTARQCFPSRDLKDYEAWLGIHDVHGRGDEKCKQVLNVSQLVYGPEGSDLVLMKLARPAVLDDFVSTIDLPNYGCTIPEKTSCSVYGWGYTGLINYDGLLRVAHLYIMGNEKCSQHHRGKVTLNESEICAGAEKIGSGPCEGDYGGPLVCEQHKMRMVLGVIVPGRGCAIPNRPGIFVRVAYYAKWIHKIILTYKVPQS

SEQ ID NO: 27 - protein, 728 aa, synthetic construct
  REGION 1..728: note = HGF Variant
MWVTKLLPALLLQHVLLHLLLLPIAIPYAEGQGKRRNTIHEFKKSAKTTLIKIDPALKIKTEKVNTADQCANRCTRSKGLPFTCKAFVFDKARKRCLWFPFNSMSSGVKKEFGHEFDLYENKDYIRDCIIGNGRSYRGTVSITKSGIKCQPWSAMIPHEHSFLPSSYRGEDLRENYCRNPRGEEGGPWCYTSDPEVRYEVCDIPQCSEVECMTCNGESYRGLMDHTESGKICQRWDHQTPHRHKFLPERYPDKGFDDNYCRNPDGQPRPWCYTLDPHTRWEYCAIKTCADNTMNDTDVPLETTECIQGQGEGYRGTVNTIWNGIPCQRWDSQYPHEHDMTPENFKCKDLRENYCRNPDGSESPWCFTTDPNIRVGYCSQIPNCDMSHGQDCYRGNGKNYMGNLSQTRSGLTCSMWDKNMEDLHRHIFWEPDASKLNENYCRNPDDDAHGPWCYTGNPLIPWDYCPISRCEGDTTPTIVNLDHPVISCAKTKQLRVVNGIPTRTNIGWMVSLRYRNKHICGGSLIKESWVLTARQCFPSRDLKDYEAWLGIHDVHGRGDEKCKQVLNVSQLVYGPEGSDLVLMKLARPAVLDDFVSTIDLPNYGCTIPEKTSCSVYGWGYTGLINYDGLLRVAHLYIMGNEKCSQHHRGKVTLNESEICAGAEKIGSGPCEGDYGGPLVCEQHKMRMVLGVIVPGRGCAIPNRPGIFVRVAYYAKWIHKIILTYKVPQS

SEQ ID NO: 28 - protein, 140 aa, Homo sapiens
FNLPPGNYKKPKLLYCSNGGHFLRILPDGTVDGTRDRSDQHIQLQLSAESVGEVYIKSTETGQYLAMDTDGLLYGSQTPNEECLFLERLEENHYNTYISKKHAEKNWFVGLKKNGSCKRGPRTHYGQKAILFLPLPVSSD

SEQ ID NO: 29 - protein, 140 aa, synthetic construct
  REGION 1..140: note = FGF1 Variant
FNLPPGNYKKPKLLYCSNGGHFLRILPNGTVDGTRDRSDQHIQLQLSAESVGEVYIKSTETGQYLAMDTDGLLYGSQTPNEECLFLERLEENHYNTYISKKHAEKNWFVGLKKNGSCKRGPRTHYGQKAIRFLPLPVSSD

SEQ ID NO: 30 - protein, 140 aa, synthetic construct
  REGION 1..140: note = FGF1 Variant
FNLPPGNYKKPKLLYCSNGGHFLRILPDGTVDGTRDRSDPHIQLQLIAESVGEVYIKSTETGQYLAMDTDGLLYGSQTPNEECLFLERLEENGYNTYISKKHAEKNWFVGLKKNGSCKRGPRTHYGQKAILFLPLPVSSD

SEQ ID NO: 31 - protein, 140 aa, synthetic construct
  REGION 1..140: note = FGF1 Variant
FNLPPGNYKKPKLLYCSNGGHFLRILPNGTVDGTRDRSDPHIQLQLIAESVGEVYIKSTETGQYLAMDTDGLLYGSQTPNEECLFLERLEENGYNTYISKKHAEKNWFVGLKKNGSCKRGPRTHYGQKAIRFLPLPVSSD

SEQ ID NO: 32 - protein, 140 aa, synthetic construct
  REGION 1..140: note = FGF1 Variant
FNLPPGNYKKPKLLYCSNGGHFLRILPDGTVDGTRDRSDQHIQLQLSAESVGEVYIKSTETGQYLAMDTDGLLYGSQTPNEECLFLERLEENHYNTYISKKHAEKNWFVGLKKNGSCKRGPRTHYGQKAIRFLPLPVSSD

SEQ ID NO: 33 - protein, 140 aa, synthetic construct
  REGION 1..140: note = FGF1 Variant
FNLPPGNYKKPKLLYCSNGGHFLRILPDGTVDGTRDRSDQHIQLQLSAESVGEVYIKSTETGQYLAMDTDGLLYGSQTPNEECLFLERLEENHYNTYISKKHAEKNWFVGLKKNGSCKRGPRTHYGQKAIKFLPLPVSSD

SEQ ID NO: 34 - protein, 31 aa, Homo sapiens
MWVTKLLPALLLQHVLLHLLLLPIAIPYAEG

SEQ ID NO: 35 - protein, 692 aa, Homo sapiens
QRKRRNTIHEFKKSAKTTLIKIDPALKIKTKKVNTADQCANRCTRNKGLPFTCKAFVFDKARKQCLWFPFNSMSSGVKKEFGHEFDLYENKDYIRNCIIGKGRSYKGTVSITKSGIKCQPWSSMIPHEHSYRGKDLQENYCRNPRGEEGGPWCFTSNPEVRYEVCDIPQCSEVECMTCNGESYRGLMDHTESGKICQRWDHQTPHRHKFLPERYPDKGFDDNYCRNPDGQPRPWCYTLDPHTRWEYCAIKTCADNTMNDTDVPLETTECIQGQGEGYRGTVNTIWNGIPCQRWDSQYPHEHDMTPENFKCKDLRENYCRNPDGSESPWCFTTDPNIRVGYCSQIPNCDMSHGQDCYRGNGKNYMGNLSQTRSGLTCSMWDKNMEDLHRHIFWEPDASKLNENYCRNPDDDAHGPWCYTGNPLIPWDYCPISRCEGDTTPTIVNLDHPVISCAKTKQLRVVNGIPTRTNIGWMVSLRYRNKHICGGSLIKESWVLTARQCFPSRDLKDYEAWLGIHDVHGRGDEKCKQVLNVSQLVYGPEGSDLVLMKLARPAVLDDFVSTIDLPNYGCTIPEKTSCSVYGWGYTGLINYDGLLRVAHLYIMGNEKCSQHHRGKVTLNESEICAGAEKIGSGPCEGDYGGPLVCEQHKMRMVLGVIVPGRGCAIPNRPGIFVRVAYYAKWIHKIILTYKVPQS

SEQ ID NO: 36 - protein, 458 aa, Homo sapiens
QRKRRNTIHEFKKSAKTTLIKIDPALKIKTKKVNTADQCANRCTRNKGLPFTCKAFVFDKARKQCLWFPFNSMSSGVKKEFGHEFDLYENKDYIRNCIIGKGRSYKGTVSITKSGIKCQPWSSMIPHEHSYRGKDLQENYCRNPRGEEGGPWCFTSNPEVRYEVCDIPQCSEVECMTCNGESYRGLMDHTESGKICQRWDHQTPHRHKFLPERYPDKGFDDNYCRNPDGQPRPWCYTLDPHTRWEYCAIKTCADNTMNDTDVPLETTECIQGQGEGYRGTVNTIWNGIPCQRWDSQYPHEHDMTPENFKCKDLRENYCRNPDGSESPWCFTTDPNIRVGYCSQIPNCDMSHGQDCYRGNGKNYMGNLSQTRSGLTCSMWDKNMEDLHRHIFWEPDASKLNENYCRNPDDDAHGPWCYTGNPLIPWDYCPISRCEGDTTPTIVNLDHPVISCAKTKQLR

SEQ ID NO: 37 - protein, 234 aa, Homo sapiens
VVNGIPTRTNIGWMVSLRYRNKHICGGSLIKESWVLTARQCFPSRDLKDYEAWLGIHDVHGRGDEKCKQVLNVSQLVYGPEGSDLVLMKLARPAVLDDFVSTIDLPNYGCTIPEKTSCSVYGWGYTGLINYDGLLRVAHLYIMGNEKCSQHHRGKVTLNESEICAGAEKIGSGPCEGDYGGPLVCEQHKMRMVLGVIVPGRGCAIPNRPGIFVRVAYYAKWIHKIILTYKVPQS